European Patent Specification EP 3 544 015 B1, published October 23, 2024. Title: SIGNAL ENCODING AND DECODING IN MULTIPLEXED BIOCHEMICAL ASSAYS. Applicant: CALIFORNIA INSTITUTE OF TECHNOLOGY. Application EP13744261.2. The sequence listing filed with the application follows.

SEQUENCE LISTING (32 sequences)

SEQ ID NO: 1 - DNA, 198 bp, Human immunodeficiency virus 1
ggaagctctattagatacaggagcagatgatacagtattagaagaaatgagtttgccaggaagatggaaaccaaaaatgatagggggaattggaggttttatcaaagtaagacagtatgatcagatactcatagaaatctgtggacataaagctataggtacagtattagtaggacctacacctgtcaacataattgg

SEQ ID NO: 2 - DNA, 26 bp, Artificial Sequence
  Description of Artificial Sequence: Synthetic primer
ggaagctctattagatacaggagcag

SEQ ID NO: 3 - DNA, 26 bp, Artificial Sequence
  Description of Artificial Sequence: Synthetic primer
ccaattatgttgacaggtgtaggtcc

SEQ ID NO: 4 - DNA, 26 bp, Artificial Sequence
  Description of Artificial Sequence: Synthetic probe
  5'6-FAM
  3'BHQ_1
tgagtttgccaggaagatggaaacca

SEQ ID NO: 5 - DNA, 199 bp, Human immunodeficiency virus 1
cagctacaaccatcccttcagacaggatcagaagaacttagatcattatataatacagtagcaaccctctattgtgtgcatcaaaggatagagataaaagacaccaaggaagctttagacaagatagaggaagagcaaaacaaaagtaagaaaaaagcacagcaagcagcagctgacacaggacacagcaatcaggtca

SEQ ID NO: 6 - DNA, 24 bp, Artificial Sequence
  Description of Artificial Sequence: Synthetic primer
cagctacaaccatcccttcagaca

SEQ ID NO: 7 - DNA, 24 bp, Artificial Sequence
  Description of Artificial Sequence: Synthetic primer
tgacctgattgctgtgtcctgtgt

SEQ ID NO: 8 - DNA, 28 bp, Artificial Sequence
  Description of Artificial Sequence: Synthetic probe
  5'6-FAM
  3'BHQ_1
agcaaccctctattgtgtgcatcaaagg

SEQ ID NO: 9 - DNA, 23 bp, Artificial Sequence
  Description of Artificial Sequence: Synthetic probe
  5'Cy3
  3'BHQ_2
aaagcacagcaagcagcagctga

SEQ ID NO: 10 - DNA, 199 bp, Plasmodium falciparum
gcctaacatggctatgacgggtaacggggaattagagttcgattccggagagggagcctgagaaatagctaccacatctaaggaaggcagcaggcgcgtaaattacccaattctaaagaagagaggtagtgacaagaaataacaatgcaaggccaatttaaaaccttcccagagtaacaattggagggcaagtctggtg

SEQ ID NO: 11 - DNA, 24 bp, Artificial Sequence
  Description of Artificial Sequence: Synthetic primer
gcctaacatggctatgacgggtaa

SEQ ID NO: 12 - DNA, 24 bp, Artificial Sequence
  Description of Artificial Sequence: Synthetic primer
caccagacttgccctccaattgtt

SEQ ID NO: 13 - DNA, 26 bp, Artificial Sequence
  Description of Artificial Sequence: Synthetic probe
  5'6-FAM
  3'BHQ_1
attccggagagggagcctgagaaata

SEQ ID NO: 14 - DNA, 26 bp, Artificial Sequence
  Description of Artificial Sequence: Synthetic probe
  5'6-ROXN
  3'BHQ_2
aaggaaggcagcaggcgcgtaaatta

SEQ ID NO: 15 - DNA, 192 bp, Herpes simplex virus 2
tcagcccatcctccttcggcagtatggagggtgtcgcggcggcgagccgccgtccccaaagacgtgcgggtcgtacacgtacacgtaccagggcggcgggcctccgacccggtacgctctcgtaaatgcttccctgctggtgccgatctgggaccgcgccgcggagacattcgagtaccagatcgaactcgg

SEQ ID NO: 16 - DNA, 25 bp, Artificial Sequence
  Description of Artificial Sequence: Synthetic primer
tcagcccatcctccttcggcagtat

SEQ ID NO: 17 - DNA, 26 bp, Artificial Sequence
  Description of Artificial Sequence: Synthetic primer
ccgagttcgatctggtactcgaatgt

SEQ ID NO: 18 - DNA, 26 bp, Artificial Sequence
  Description of Artificial Sequence: Synthetic probe
  5'6-FAM
  3'BHQ_1
aaagacgtgcgggtcgtacacgtaca

SEQ ID NO: 19 - DNA, 25 bp, Artificial Sequence
  Description of Artificial Sequence: Synthetic probe
  5'Cy5
  3'3IAbRQSp
taaatgcttccctgctggtgccgat

SEQ ID NO: 20 - DNA, 200 bp, Mycobacterium tuberculosis
gagtgcaaagacaaggacatgacgtacgcggccccgctgttcgtcacggccgagttcatcaacaacaacaccggcgagatcaagagccagacggtgttcatgggtgacttcccgatgatgaccgagaagggcaccttcatcatcaacggcaccgagcgcgtcgtggtcagccagctggtccgctcgcccggtgtgtactt

SEQ ID NO: 21 - DNA, 24 bp, Artificial Sequence
  Description of Artificial Sequence: Synthetic primer
gagtgcaaagacaaggacatgacg

SEQ ID NO: 22 - DNA, 19 bp, Artificial Sequence
  Description of Artificial Sequence: Synthetic primer
aagtacacaccgggcgagc

SEQ ID NO: 23 - DNA, 25 bp, Artificial Sequence
  Description of Artificial Sequence: Synthetic probe
  5'6-FAM
  3'BHQ_1
cgctgttcgtcacggccgagttcat

SEQ ID NO: 24 - DNA, 26 bp, Artificial Sequence
  Description of Artificial Sequence: Synthetic probe
  5'Cy3
  3'BHQ_2
agatcaagagccagacggtgttcatg

SEQ ID NO: 25 - DNA, 25 bp, Artificial Sequence
  Description of Artificial Sequence: Synthetic probe
  5'Cy5
  3'IAbRQSp
aagggcaccttcatcatcaacggca

SEQ ID NO: 26 - DNA, 200 bp, Dengue virus 3
atgccaactgtgattgagcacttagaaagactacaaaggaaacatggaggaatgcttgtgagaaatccactctcacgaaactccacgcacgaaatgtattggatatccaatggtacaggcaacatcgtctcattcacaatgacacacaggagacccaccatagagaaagatgtggatttaggagcaggaacccgacatgt

SEQ ID NO: 27 - DNA, 22 bp, Artificial Sequence
  Description of Artificial Sequence: Synthetic primer
atgccaactgtgattgagcact

SEQ ID NO: 28 - DNA, 24 bp, Artificial Sequence
  Description of Artificial Sequence: Synthetic primer
acatgtcgggttcctgctcctaaa

SEQ ID NO: 29 - DNA, 29 bp, Artificial Sequence
  Description of Artificial Sequence: Synthetic probe
  5'6-FAM
  3'BHQ_1
acaaaggaaacatggaggaatgcttgtga

SEQ ID NO: 30 - DNA, 26 bp, Artificial Sequence
  Description of Artificial Sequence: Synthetic probe
  5'Cy3
  3'BHQ_2
actctcacgaaactccacgcacgaaa

SEQ ID NO: 31 - DNA, 26 bp, Artificial Sequence
  Description of Artificial Sequence: Synthetic probe
  5'6-ROXN
  3'BHQ_2
acaatgacacacaggagacccaccat

SEQ ID NO: 32 - DNA, 28 bp, Artificial Sequence
  Description of Artificial Sequence: Synthetic probe
  5'Cy5
  3'IAbRQSp
ggatatccaatggtacaggcaacatcgt